European Patent Application EP 4 289 867 A1, published December 13, 2023. Title: CHIMERIC ANTIGEN RECEPTOR WITH ENDOGENOUS PROTEIN MOLECULE REPLACING SINGLE DOMAIN ANTIBODY. Applicant: ZHEJIANG UNIVERSITY. The sequence listing filed with the application follows.

SEQUENCE LISTING (28 sequences)

SEQ ID NO: 1 - protein, 115 aa, Homo sapiens
IPTEIPTSALVKETLALLSTHRTLLIANETLRIPVPVHKNHQLCTEEIFQGIGTLESQTVQGGTVERLFKNLSLIKKYIDGQKKKCGEERRRVNQFLDYLQEFLGVMNTEWIIES

SEQ ID NO: 2 - protein, 113 aa, Mus musculus
MEIPMSTVVKETLTQLSAHRALLTSNETMRLPVPTHKNHQLCIGEIFQGLDILKNQTVRGGTVEMLFQNLSLIKKYIDRQKEKCGEERRRTRQFLDYLQEFLGVMSTEWAMEG

SEQ ID NO: 3 - protein, 411 aa, Homo sapiens
SNELHQVPSNCDCLNGGTCVSNKYFSNIHWCNCPKKFGGQHCEIDKSKTCYEGNGHFYRGKASTDTMGRPCLPWNSATVLQQTYHAHRSDALQLGLGKHNYCRNPDNRRRPWCYVQVGLKLLVQECMVHDCADGKKPSSPPEELKFQCGQKTLRPRFKIIGGEFTTIENQPWFAAIYRRHRGGSVTYVCGGSLISPCWVISATHCFIDYPKKEDYIVYLGRSRLNSNTQGEMKFEVENLILHKDYSADTLAHHNDIALLKIRSKEGRCAQPSRTIQTICLPSMYNDPQFGTSCEITGFGKENSTDYLYPEQLKMTVVKLISHRECQQPHYYGSEVTTKMLCAADPQWKTDSCQGDSGGPLVCSLQGRMTLTGIVSWGRGCALKDKPGVYTRVSHFLPWIRSHTKEENGLAL

SEQ ID NO: 4 - protein, 74 aa, Homo sapiens
GPASVPTTCCFNLANRKIPLQRLESYRRITSGKCPQKAVIFKTKLAKDICADPKKKWVQDSMKYLDQKSPTPKP

SEQ ID NO: 5 - protein, 93 aa, Homo sapiens
VVIPSPCCMFFVSKRIPENRVVSYQLSSRSTCLKAGVIFTTKKGQQFCGDPKQEWVQRYMKNLDAKQKKASPRARAVAVKGPVQRYPGNQTTC

SEQ ID NO: 6 - protein, 356 aa, artificial sequence
  the amino acid sequence of said ECAR
MALPVTALLLPLALLLHAIPTEIPTSALVKETLALLSTHRTLLIANETLRIPVPVHKNHQLCTEEIFQGIGTLESQTVQGGTVERLFKNLSLIKKYIDGQKKKCGEERRRVNQFLDYLQEFLGVMNTEWIIESRAAAIEVMYPPPYLDNEKSNGTIIHVKGKHLCPSPLFPGPSKPFWVLVVVGGVLACYSLLVTVAFIIFWVRSKRSRLLHSDYMNMTPRRPGPTRKHYQPYAPPRDFAAYRSRVKFSRSADAPAYQQGQNQLYNELNLGRREEYDVLDKRRGRDPEMGGKPRRKNPQEGLYNELQKDKMAEAYSEIGMKGERRRGKGHDGLYQGLSTATKDTYDALHMQALPPR

SEQ ID NO: 7 - protein, 370 aa, artificial sequence
  the amino acid sequence of said ECAR
MASPLTRFLSLNLLLLGESIILGSGEAMEIPMSTVVKETLTQLSAHRALLTSNETMRLPVPTHKNHQLCIGEIFQGLDILKNQTVRGGTVEMLFQNLSLIKKYIDRQKEKCGEERRRTRQFLDYLQEFLGVMSTEWAMEGRAAASTTTKPVLRTPSPVHPTGTSQPQRPEDCRPRGSVKGTGLDFACDIYIWAPLAGICVALLLSLIITLICYNSRRNRLLQSDYMNMTPRRPGLTRKPYQPYAPARDFAAYRPRAKFSRSAETAANLQDPNQLYNELNLGRREEYDVLEKKRARDPEMGGKQQRRRNPQEGVYNALQKDKMAEAYSEIGTKGERRRGKGHDGLYQGLSTATKDTYDALHMQTLAPRGSG

SEQ ID NO: 8 - protein, 661 aa, artificial sequence
  the amino acid sequence of said ECAR
MALPVTALLLPLALLLHAYPYDVPDYASNELHQVPSNCDCLNGGTCVSNKYFSNIHWCNCPKKFGGQHCEIDKSKTCYEGNGHFYRGKASTDTMGRPCLPWNSATVLQQTYHAHRSDALQLGLGKHNYCRNPDNRRRPWCYVQVGLKLLVQECMVHDCADGKKPSSPPEELKFQCGQKTLRPRFKIIGGEFTTIENQPWFAAIYRRHRGGSVTYVCGGSLISPCWVISATHCFIDYPKKEDYIVYLGRSRLNSNTQGEMKFEVENLILHKDYSADTLAHHNDIALLKIRSKEGRCAQPSRTIQTICLPSMYNDPQFGTSCEITGFGKENSTDYLYPEQLKMTVVKLISHRECQQPHYYGSEVTTKMLCAADPQWKTDSCQGDSGGPLVCSLQGRMTLTGIVSWGRGCALKDKPGVYTRVSHFLPWIRSHTKEENGLALRAAAIEVMYPPPYLDNEKSNGTIIHVKGKHLCPSPLFPGPSKPFWVLVVVGGVLACYSLLVTVAFIIFWVRSKRSRLLHSDYMNMTPRRPGPTRKHYQPYAPPRDFAAYRSRVKFSRSADAPAYQQGQNQLYNELNLGRREEYDVLDKRRGRDPEMGGKPRRKNPQEGLYNELQKDKMAEAYSEIGMKGERRRGKGHDGLYQGLSTATKDTYDALHMQALPPR

SEQ ID NO: 9 - protein, 324 aa, artificial sequence
  the amino acid sequence of said ECAR
MALPVTALLLPLALLLHAYPYDVPDYAGPASVPTTCCFNLANRKIPLQRLESYRRITSGKCPQKAVIFKTKLAKDICADPKKKWVQDSMKYLDQKSPTPKPRAAAIEVMYPPPYLDNEKSNGTIIHVKGKHLCPSPLFPGPSKPFWVLVVVGGVLACYSLLVTVAFIIFWVRSKRSRLLHSDYMNMTPRRPGPTRKHYQPYAPPRDFAAYRSRVKFSRSADAPAYQQGQNQLYNELNLGRREEYDVLDKRRGRDPEMGGKPRRKNPQEGLYNELQKDKMAEAYSEIGMKGERRRGKGHDGLYQGLSTATKDTYDALHMQALPPR

SEQ ID NO: 10 - protein, 343 aa, artificial sequence
  the amino acid sequence of said ECAR
MALPVTALLLPLALLLHAYPYDVPDYAVVIPSPCCMFFVSKRIPENRVVSYQLSSRSTCLKAGVIFTTKKGQQFCGDPKQEWVQRYMKNLDAKQKKASPRARAVAVKGPVQRYPGNQTTCRAAAIEVMYPPPYLDNEKSNGTIIHVKGKHLCPSPLFPGPSKPFWVLVVVGGVLACYSLLVTVAFIIFWVRSKRSRLLHSDYMNMTPRRPGPTRKHYQPYAPPRDFAAYRSRVKFSRSADAPAYQQGQNQLYNELNLGRREEYDVLDKRRGRDPEMGGKPRRKNPQEGLYNELQKDKMAEAYSEIGMKGERRRGKGHDGLYQGLSTATKDTYDALHMQALPPR

SEQ ID NO: 11 - DNA, 1068 bp, artificial sequence
  the nucleotide sequence of said ECAR
atggctctcccagtgactgccctactgcttcccctagcgcttctcctgcatgcaatccccacagaaattcccacaagtgcattggtgaaagagaccttggcactgctttctactcatcgaactctgctgatagccaatgagactctgaggattcctgttcctgtacataaaaatcaccaactgtgcactgaagaaatctttcagggaataggcacactggagagtcaaactgtgcaagggggtactgtggaaagactattcaaaaacttgtccttaataaagaaatacattgacggccaaaaaaaaaagtgtggagaagaaagacggagagtaaaccaattcctagactacctgcaagagtttcttggtgtaatgaacaccgagtggataatagaaagtcgggcggccgcaattgaagttatgtatcctcctccttacctagacaatgagaagagcaatggaaccattatccatgtgaaagggaaacacctttgtccaagtcccctatttcccggaccttctaagcccttttgggtgctggtggtggttggtggagtcctggcttgctatagcttgctagtaacagtggcctttattattttctgggtgaggagtaagaggagcaggctcctgcacagtgactacatgaacatgactccccgccgccccgggcccacccgcaagcattaccagccctatgccccaccacgcgacttcgcagcctatcgctccagagtgaagttcagcaggagcgcagacgcccccgcgtaccagcagggccagaaccagctctataacgagctcaatctaggacgaagagaggagtacgatgttttggacaagagacgtggccgggaccctgagatggggggaaagccgagaaggaagaaccctcaggaaggcctgtacaatgaactgcagaaagataagatggcggaggcctacagtgagattgggatgaaaggcgagcgccggaggggcaaggggcacgatggcctttaccagggtctcagtacagccaccaaggacacctacgacgcccttcacatgcaggccctgccccctcgc

SEQ ID NO: 12 - DNA, 1110 bp, artificial sequence
  the nucleotide sequence of said ECAR
atggcctcaccgttgacccgctttctgtcgctgaacctgctgctgctgggtgagtcgattatcctggggagtggagaagctatggagattcccatgagcacagtggtgaaagagaccttgacacagctgtccgctcaccgagctctgttgacaagcaatgagacgatgaggcttcctgtccctactcataaaaatcaccagctatgcattggagaaatctttcaggggctagacatactgaagaatcaaactgtccgtgggggtactgtggaaatgctattccaaaacctgtcattaataaagaaatacattgaccgccaaaaagagaagtgtggcgaggagagacggaggacgaggcagttcctggattacctgcaagagttccttggtgtgatgagtacagagtgggcaatggaaggccgggcggccgcatctactactaccaagccagtgctgcgaactccctcacctgtgcaccctaccgggacatctcagccccagagaccagaagattgtcggccccgtggctcagtgaaggggaccggattggacttcgcctgtgatatttacatctgggcacccttggccggaatctgcgtggcccttctgctgtccttgatcatcactctcatctgctacaatagtagaaggaacagactccttcaaagtgactacatgaacatgactccccggaggcctgggctcactcgaaagccttaccagccctacgcccctgccagagactttgcagcgtaccgccccagagcaaaattcagcaggagtgcagagactgctgccaacctgcaggaccccaaccagctctacaatgagctcaatctagggcgaagagaggaatatgacgtcttggagaagaagcgggctcgggatccagagatgggaggcaaacagcagaggaggaggaacccccaggaaggcgtatacaatgcactgcagaaagacaagatggcagaagcctacagtgagatcggcacaaaaggcgagaggcggagaggcaaggggcacgatggcctttaccagggtctcagcactgccaccaaggacacctatgatgccctgcatatgcagaccctggcccctcgcggatctgga

SEQ ID NO: 13 - DNA, 1983 bp, artificial sequence
  the nucleotide sequence of said ECAR
atggctctcccagtgactgccctactgcttcccctagcgcttctcctgcatgcatatccatacgacgttccggactacgcaagcaatgaacttcatcaagttccatcgaactgtgactgtctaaatggaggaacatgtgtgtccaacaagtacttctccaacattcactggtgcaactgcccaaagaaattcggagggcagcactgtgaaatagataagtcaaaaacctgctatgaggggaatggtcacttttaccgaggaaaggccagcactgacaccatgggccggccctgcctgccctggaactctgccactgtccttcagcaaacgtaccatgcccacagatctgatgctcttcagctgggcctggggaaacataattactgcaggaacccagacaaccggaggcgaccctggtgctatgtgcaggtgggcctaaagctgcttgtccaagagtgcatggtgcatgactgcgcagatggaaaaaagccctcctctcctccagaagaattaaaatttcagtgtggccaaaagactctgaggccccgctttaagattattgggggagaattcaccaccatcgagaaccagccctggtttgcggccatctacaggaggcaccgggggggctctgtcacctacgtgtgtggaggcagcctcatcagcccttgctgggtgatcagcgccacacactgcttcattgattacccaaagaaggaggactacatcgtctacctgggtcgctcaaggcttaactccaacacgcaaggggagatgaagtttgaggtggaaaacctcatcctacacaaggactacagcgctgacacgcttgctcaccacaacgacattgccttgctgaagatccgttccaaggagggcaggtgtgcgcagccatcccggactatacagaccatctgcctgccctcgatgtataacgatccccagtttggcacaagctgtgagatcactggctttggaaaagagaattctaccgactatctctatccggagcagctgaaaatgactgttgtgaagctgatttcccaccgggagtgtcagcagccccactattacggctctgaagtcaccaccaaaatgctgtgtgctgctgacccacagtggaaaacagattcctgccagggagactcagggggacccctcgtctgttccctccaaggccgcatgactttgactggaattgtgagctggggccgtggatgtgccctgaaggacaagccaggcgtctacacgagagtctcacacttcttaccctggatccgcagtcacaccaaggaagagaatggcctggccctccgggcggccgcaattgaagttatgtatcctcctccttacctagacaatgagaagagcaatggaaccattatccatgtgaaagggaaacacctttgtccaagtcccctatttcccggaccttctaagcccttttgggtgctggtggtggttggtggagtcctggcttgctatagcttgctagtaacagtggcctttattattttctgggtgaggagtaagaggagcaggctcctgcacagtgactacatgaacatgactccccgccgccccgggcccacccgcaagcattaccagccctatgccccaccacgcgacttcgcagcctatcgctccagagtgaagttcagcaggagcgcagacgcccccgcgtaccagcagggccagaaccagctctataacgagctcaatctaggacgaagagaggagtacgatgttttggacaagagacgtggccgggaccctgagatggggggaaagccgagaaggaagaaccctcaggaaggcctgtacaatgaactgcagaaagataagatggcggaggcctacagtgagattgggatgaaaggcgagcgccggaggggcaaggggcacgatggcctttaccagggtctcagtacagccaccaaggacacctacgacgcccttcacatgcaggccctgccccctcgc

SEQ ID NO: 14 - DNA, 972 bp, artificial sequence
  the nucleotide sequence of said ECAR
atggctctcccagtgactgccctactgcttcccctagcgcttctcctgcatgcatatccatacgacgttccggactacgcagggccagcttctgtcccaaccacctgctgctttaacctggccaataggaagataccccttcagcgactagagagctacaggagaatcaccagtggcaaatgtccccagaaagctgtgatcttcaagaccaaactggccaaggatatctgtgccgaccccaagaagaagtgggtgcaggattccatgaagtatctggaccaaaaatctccaactccaaagccacgggcggccgcaattgaagttatgtatcctcctccttacctagacaatgagaagagcaatggaaccattatccatgtgaaagggaaacacctttgtccaagtcccctatttcccggaccttctaagcccttttgggtgctggtggtggttggtggagtcctggcttgctatagcttgctagtaacagtggcctttattattttctgggtgaggagtaagaggagcaggctcctgcacagtgactacatgaacatgactccccgccgccccgggcccacccgcaagcattaccagccctatgccccaccacgcgacttcgcagcctatcgctccagagtgaagttcagcaggagcgcagacgcccccgcgtaccagcagggccagaaccagctctataacgagctcaatctaggacgaagagaggagtacgatgttttggacaagagacgtggccgggaccctgagatggggggaaagccgagaaggaagaaccctcaggaaggcctgtacaatgaactgcagaaagataagatggcggaggcctacagtgagattgggatgaaaggcgagcgccggaggggcaaggggcacgatggcctttaccagggtctcagtacagccaccaaggacacctacgacgcccttcacatgcaggccctgccccctcgc

SEQ ID NO: 15 - DNA, 1029 bp, artificial sequence
  the nucleotide sequence of said ECAR
atggctctcccagtgactgccctactgcttcccctagcgcttctcctgcatgcatatccatacgacgttccggactacgcagtggtcatcccctctccctgctgcatgttctttgtttccaagagaattcctgagaaccgagtggtcagctaccagctgtccagcaggagcacatgcctcaaggcaggagtgatcttcaccaccaagaagggccagcagttctgtggcgaccccaagcaggagtgggtccagaggtacatgaagaacctggacgccaagcagaagaaggcttcccctagggccagggcagtggctgtcaagggccctgtccagagatatcctggcaaccaaaccacctgccgggcggccgcaattgaagttatgtatcctcctccttacctagacaatgagaagagcaatggaaccattatccatgtgaaagggaaacacctttgtccaagtcccctatttcccggaccttctaagcccttttgggtgctggtggtggttggtggagtcctggcttgctatagcttgctagtaacagtggcctttattattttctgggtgaggagtaagaggagcaggctcctgcacagtgactacatgaacatgactccccgccgccccgggcccacccgcaagcattaccagccctatgccccaccacgcgacttcgcagcctatcgctccagagtgaagttcagcaggagcgcagacgcccccgcgtaccagcagggccagaaccagctctataacgagctcaatctaggacgaagagaggagtacgatgttttggacaagagacgtggccgggaccctgagatggggggaaagccgagaaggaagaaccctcaggaaggcctgtacaatgaactgcagaaagataagatggcggaggcctacagtgagattgggatgaaaggcgagcgccggaggggcaaggggcacgatggcctttaccagggtctcagtacagccaccaaggacacctacgacgcccttcacatgcaggccctgccccctcgc

SEQ ID NO: 16 - protein, 21 aa, Homo sapiens
MALPVTALLLPLALLLHAARP

SEQ ID NO: 17 - protein, 27 aa, Mus musculus
MASPLTRFLSLNLLLLGESIILGSGEA

SEQ ID NO: 18 - protein, 39 aa, Homo sapiens
IEVMYPPPYLDNEKSNGTIIHVKGKHLCPSPLFPGPSKP

SEQ ID NO: 19 - protein, 45 aa, Homo sapiens
TTTPAPRPPTPAPTIASQPLSLRPEACRPAAGGAVHTRGLDFACD

SEQ ID NO: 20 - protein, 46 aa, Mus musculus
STTTKPVLRTPSPVHPTGTSQPQRPEDCRPRGSVKGTGLDFACDIY

SEQ ID NO: 21 - protein, 27 aa, Homo sapiens
FWVLVVVGGVLACYSLLVTVAFIIFWV

SEQ ID NO: 22 - protein, 21 aa, Homo sapiens
IYIWAPLAGTCGVLLLSLVIT

SEQ ID NO: 23 - protein, 21 aa, Mus musculus
IWAPLAGICVALLLSLIITLI

SEQ ID NO: 24 - protein, 41 aa, Homo sapiens
RSKRSRLLHSDYMNMTPRRPGPTRKHYQPYAPPRDFAAYRS

SEQ ID NO: 25 - protein, 42 aa, Homo sapiens
KRGRKKLLYIFKQPFMRPVQTTQEEDGCSCRFPEEEEGGCEL

SEQ ID NO: 26 - protein, 41 aa, Mus musculus
NSRRNRLLQSDYMNMTPRRPGLTRKPYQPYAPARDFAAYRP

SEQ ID NO: 27 - protein, 112 aa, Homo sapiens
RVKFSRSADAPAYKQGQNQLYNELNLGRREEYDVLDKRRGRDPEMGGKPRRKNPQEGLYNELQKDKMAEAYSEIGMKGERRRGKGHDGLYQGLSTATKDTYDALHMQALPPR

SEQ ID NO: 28 - protein, 113 aa, Mus musculus
RAKFSRSAETAANLQDPNQLYNELNLGRREEYDVLEKKRARDPEMGGKQQRRRNPQEGVYNALQKDKMAEAYSEIGTKGERRRGKGHDGLYQGLSTATKDTYDALHMQTLAPR